European Patent Application EP 4 509 528 A1, published February 19, 2025. Title: MONOCLONAL ANTIBODIES AGAINST VETERINARY PROGASTRIN-LIKE MOLECULES AND THEIR USES. Applicant: Barrelman BioSciences LLC. The sequence listing filed with the application follows.

SEQUENCE LISTING (103 sequences)

SEQ ID NO: 1 - protein, 16 aa, synthetic construct
SWKPRSRLQDAPSGPG

SEQ ID NO: 2 - protein, 29 aa, synthetic construct
QGPWMEEEEAAYGWMDFGRRSAEEGDQRP

SEQ ID NO: 3 - protein, 17 aa, synthetic construct
SWKPRSRLQDAPSGPGC

SEQ ID NO: 4 - protein, 30 aa, synthetic construct
CQGPWMEEEEAAYGWMDFGRRSAEEGDQRP

SEQ ID NO: 5 - protein, 14 aa, synthetic construct
SWKPRSQQPDAPLG

SEQ ID NO: 6 - protein, 26 aa, synthetic construct
QGPWLEEEEEAYGWMDFGRRSAEDEN

SEQ ID NO: 7 - DNA, 42 bp, synthetic construct
  source 1..42: mol_type = other DNA
atggagactgggctgcgctggcttctcctggtcgctgtgctc

SEQ ID NO: 8 - DNA, 41 bp, synthetic construct
  source 1..41: mol_type = other DNA
cacccagctccacggtcaccctgggttgtcttgtgaaggga

SEQ ID NO: 9 - DNA, 58 bp, synthetic construct
  source 1..58: mol_type = other DNA
atggacacgagggcccccactcagctgctggggctcctgctgctctggctcccaggtg

SEQ ID NO: 10 - DNA, 50 bp, synthetic construct
  source 1..50: mol_type = other DNA
tactgtcctcatcttcccaccagctgctgatcaggtggcaactggaacag

SEQ ID NO: 11 - protein, 83 aa, Mammal
SWKPRSRLQDAPSGPGANRGLEPHGLDQLGPASHHRRQLGLQGPPQLVADLSKKQGPWMEEEEAAYGWMDFGRRSAEEGDQRP

SEQ ID NO: 12 - DNA, 401 bp, synthetic construct
  source 1..401: mol_type = other DNA
aaaggtgtccagtgtcagtcgctggaggagtccgagggaggtctcttcaagccaacggataccctgacactcacctgcacagtctctggattctccctcattagctatggagtgagctgggtccgccaggctccagggaaggggctggaatggatcggaggcatttggcctggtgctagcacgtactacgcgagctgggcgaaaagccgatccaccatcaccagaaacaccaacctgaacacggtgaccctgaaaatgaccagtctgacagccgcggacacggccacctatttctgtgcgaggaatagtgttggttggctctggggcccaggcaccctggtcaccgtctcctcagggcaacctaaggctccatcagtcttcccactggccccctgctgcgg

SEQ ID NO: 13 - DNA, 413 bp, synthetic construct
  source 1..413: mol_type = other DNA
aaaggtgtccagtgtcagtcgctggaggagtccgggggtcgcctggtcaagcctgacgaaaccctgacactcacctgcacagtctctggaatcgacctcagtagcaatgcaatgaactgggtccgccaggctccagggaacgggctggagtggatcggagccattgatcgtggtggtgacacatactacgcgagctgggcgagaagccgatccaccatcaccagagacaccaacctgaacacggtgactctgaaaatgaccagtctgacagccgcggacacggccacctatttctgtgcgagaggtgcttttgcttatcctgaggctggcatctggggcccaggcaccctggtcaccgtctcctcagggcaacctaaggctccatcagtcttcccactggccccctgctgcgg

SEQ ID NO: 14 - DNA, 371 bp, synthetic construct
  source 1..371: mol_type = other DNA
aggtgccacatttgcccaagtgctgacccagtctgcatcgcccgtgtctgcagctgtgggaggcacagtcaccatcaattgccaggccagtcagagtatttataagaacaactacttatcctggtatcaccagaaaccagggcagcctcccaagctcctgatctatgatgcatccgatctggcatctggggtcccatcgcggttcagtggcagtggatctgggacacagttcactctcaccatcagcggcgtgcagtgtgaagatgctgccacttactactgtcaaggcgaatttagttgtagtagtgctgattgttttgctttcggcggagggaccgaggtggtggtcaaaggtgatccagttgcaccta

SEQ ID NO: 15 - DNA, 356 bp, synthetic construct
  source 1..356: mol_type = other DNA
aggtgccacatttgcgcaagtgctgacccagactccagcctccgtgtctgcacctgtgggaggcacagtcaccatcagttgccagtccagtgagagtgtttataacaacaacttagcctggtttcagcagaaaccagggcagcctcccaagctcctgatctatgatgcatccgatctggcatctggggtcccatcgcggttcaagggcagtggatctgggacacagttcactcttaccatcagcgacctggagtgtgacgatgctgccacttactactgtgcaggcggttatagtgatgctaatgctttcggcggagggaccgagctggtggtcaaaggtgatccagttgcaccta

SEQ ID NO: 16 - DNA, 407 bp, synthetic construct
  source 1..407: mol_type = other DNA
aaaggtgtccagtgtcagtcggtggaggagtccaggggaggtctcttcaagccaacggagcccctgacactcacctgcacagcctctggattcaccatcagtagctaccacatgggctgggtccgccagactccagggaagcagctggagtggatcgggtggattggtagtagtggtgccacatactacgcgagctgggcgacaagccggtccaccatcaccagaaacaccaacgacaacacggtgactctgaaaatgaccagtctgacagccgcggacacggccacctatttctgtgcgagaagtggttggggtagttttgacatctggggcccaggcgccctggtcaccgtctcctcagggcaacctaaggctccatcagtcttcccactggccccctgctgcgg

SEQ ID NO: 17 - DNA, 407 bp, synthetic construct
  source 1..407: mol_type = other DNA
aaaggtgtccagtgtcagtcggtgaaggagtccgagggaggtctcttcaagccaacggagcccctgacactcacctgcacagtctctggattctccctcagtagcgacaacatgggctgggtccgccagactccagggaagcagctggagtggatcgggtggattggtagtagtggtagcgcatactacgcgaggtgggcgaaaagccggtccaccatcaccagaaacaccaacgagaacacggtgactctgaaaatgaccagtctgacagccgcggacacggccacctatttctgtgcgagaagtggttggggtagttttgacatatggggcccaggcaccctggtcaccgtctcctcagggcaacctaaggctccatcagtcttcccactggccccctgctgcgg

SEQ ID NO: 18 - DNA, 362 bp, synthetic construct
  source 1..362: mol_type = other DNA
aggtgccacatttgcgcaagtgctgacccagactccagcctccgtgtctgccgctgtgggaggcacagtcaccatcaactgccagtccagtcagagtgtttataataacgaccgcttagcctggtttcagcagaaaccagggcagcctcccaagctcctgatctatctggcatccactctggcatctggggtcccatcgcggttcaaaggcagtggatctgggacacagttcactctcacaatcggcgaagtacagtgtgacgatgctgccacttactactgtcaaagctactataatggttatatttttggtttcggcggagggaccgaggtggtggtcaaaggtgatccagttgcaccta

SEQ ID NO: 19 - DNA, 362 bp, synthetic construct
  source 1..362: mol_type = other DNA
aggtgccacatttgcgcaagtgctgacccagactccatcccccgtgtctgcagctgtgggaagcacagtcaccatcagttgccagtccagtcagagtgtttatagtaacaaccgcttagcctggtttcaacagaaaccagggcagcctcccaagctcctgatctatctggcatccactctggcatctggggtcccatcgcggttcaaaggcagtggatctgggacacagttcactctcacaatcagcgaagtacagtgtgacgatgctgccacttactactgtcaaggctattatagtggttatatttttggtttcggcggagggaccgaggtggtagtcaaaggtgatccagttgcaccta

SEQ ID NO: 20 - DNA, 1368 bp, synthetic construct
  source 1..1368: mol_type = other DNA
atggagactgggctgcgctggcttctcctggtcgctgtgctcaaaggtgtccagtgtcagtcgctggaggagtccgagggaggtctcttcaagccaacggataccctgacactcacctgcacagtctctggattctccctcattagctatggagtgagctgggtccgccaggctccagggaaggggctggaatggatcggaggcatttggcctggtgctagcacgtactacgcgagctgggcgaaaagccgatccaccatcaccagaaacaccaacctgaacacggtgaccctgaaaatgaccagtctgacagccgcggacacggccacctatttctgtgcgaggaatagtgttggttggctctggggcccaggcaccctggtcaccgtctcctcagggcaacctaaggctccatcagtcttcccactggccccctgctgcggggacacacccagctccacggtcaccctgggttgtcttgtgaagggatacctcccggaacccgtgaccgtgacctggaactccggcaccctgaccaatggagtgcggaccttcccgagcgtcaggcagtcctccgggttgtacagcttgtctagcgtggtgtccgtgacgtcgtcaagccagcctgtgacttgcaatgtggcccatccggccaccaacaccaaggtcgacaagaccgtggcgccttccacctgttccaagcccacttgcccgccgcctgagctcctgggaggaccgtccgtgttcatcttccctccaaaacccaaggataccctgatgattagccgcactcccgaagtcacttgcgtggtcgtggacgtgtcgcaggacgatcctgaggtgcagttcacttggtacatcaacaacgaacaagtccggacagctagaccaccgctgcgcgagcagcagttcaactcaactatccgggtggtgtccaccctgccgatcgcgcatcaggattggctgcgggggaaggagttcaagtgcaaagtccacaacaaggccctgcccgcccccatcgaaaagaccatctccaaggctcggggccagcctctggagcccaaagtgtacaccatgggcccgcctcgcgaggagctctcctcacgctcggtgtcgctgacttgcatgattaacggcttctacccttccgacatctccgtggaatgggagaagaacggaaaagccgaagataactacaagaccacgcccgccgtgctggactccgacggaagctatttcctgtactccaagctctccgtccccacttcggaatggcagaggggggacgtgttcacttgctccgtgatgcacgaggcactccacaaccactacacccaaaagagcatttcgcggtcacctggcaagtaa

SEQ ID NO: 21 - DNA, 1524 bp, synthetic construct
  source 1..1524: mol_type = other DNA
atggagactgggctgcgctggcttctcctggtcgctgtgctcaaaggtgtccagtgtcagtcgctggaggagtccgggggtcgcctggtcaagcctgacgaaaccctgacactcacctgcacagtctctggaatcgacctcagtagcaatgcaatgaactgggtccgccaggctccagggaacgggctggagtggatcggagccattgatcgtggtggtgacacatactacgcgagctgggcgagaagccgatccaccatcaccagagacaccaacctgaacacggtgactctgaaaatgaccagtctgacagccgcggacacggccacctatttctgtgcgagaggtgcttttgcttatcctgaggctggcatctggggcccaggcaccctggtcaccgtctcctcagggcaacctaaggctccatcagtcttcccactggccccctgctgcggggacacacccagctccacggtcaccctgggttgtcttgtgaagggatacctcccggaacccgtgaccgtgacctggaactccggcaccctgaccaatggagtgcggaccttcccgagcgtcaggcagtcctccgggttgtacagcttgtctagcgtggtgtccgtgacgtcgtcaagccagcctgtgacttgcaatgtggcccatccggccaccaacaccaaggtcgacaagaccgtggcgccttccacctgttccaagcccacttgcccgccgcctgagctcctgggaggaccgtccgtgttcatcttccctccaaaacccaaggataccctgatgattagccgcactcccgaagtcacttgcgtggtcgtggacgtgtcgcaggacgatcctgaggtgcagttcacttggtacatcaacaacgaacaagtccggacagctagaccaccgctgcgcgagcagcagttcaactcaactatccgggtggtgtccaccctgccgatcgcgcatcaggattggctgcgggggaaggagttcaagtgcaaagtccacaacaaggccctgcccgcccccatcgaaaagaccatctccaaggctcggggccagcctctggagcccaaagtgtacaccatgggcccgcctcgcgaggagctctcctcacgctcggtgtcgctgacttgcatgattaacggcttctacccttccgacatctccgtggaatgggagaagaacggaaaagccgaagataactacaagaccacgcccgccgtgctggactccgacggaagctatttcctgtactccaagctctccgtccccacttcggaatggcagaggggggacgtgttcacttgctccgtgatgcacgaggcactccacaaccactacacccaaaagagcatttcgcggtcacctggcaagtaatcttccctccaaaacccaaggataccctgatgattagccgcactcccgaagtcacttgcgtggtcgtggncgtgtcgcnnncgatcctgaggtgcagttcacttggtacatcaacaacgaacaagtccnggacagctagaccan

SEQ ID NO: 22 - DNA, 720 bp, synthetic construct
  source 1..720: mol_type = other DNA
atggacacgagggcccccactcagctgctggggctcctgctgctctggctcccaggtgccacatttgcccaagtgctgacccagtctgcatcgcccgtgtctgcagctgtgggaggcacagtcaccatcaattgccaggccagtcagagtatttataagaacaactacttatcctggtatcaccagaaaccagggcagcctcccaagctcctgatctatgatgcatccgatctggcatctggggtcccatcgcggttcagtggcagtggatctgggacacagttcactctcaccatcagcggcgtgcagtgtgaagatgctgccacttactactgtcaaggcgaatttagttgtagtagtgctgattgttttgctttcggcggagggaccgaggtggtggtcaaaggtgatccagttgcacctactgtcctcatcttcccaccagctgctgatcaggtggcaactggaacagtcaccatcgtgtgcgtggctaacaagtacttcccggacgtgaccgtgacctgggaagtcgacggaaccactcagaccactggtatcgagaacagcaagacgccccagaactccgccgattgtacttataacctgtcctccacactgaccctcacctcgacccagtacaattcccacaaggagtacacttgcaaagtcacccagggaaccacttcagtggtgcagagcttcaaccggggggattgctga

SEQ ID NO: 23 - DNA, 705 bp, synthetic construct
  source 1..705: mol_type = other DNA
atggacacgagggcccccactcagctgctggggctcctgctgctctggctcccaggtgccacatttgcgcaagtgctgacccagactccagcctccgtgtctgcacctgtgggaggcacagtcaccatcagttgccagtccagtgagagtgtttataacaacaacttagcctggtttcagcagaaaccagggcagcctcccaagctcctgatctatgatgcatccgatctggcatctggggtcccatcgcggttcaagggcagtggatctgggacacagttcactcttaccatcagcgacctggagtgtgacgatgctgccacttactactgtgcaggcggttatagtgatgctaatgctttcggcggagggaccgagctggtggtcaaaggtgatccagttgcacctactgtcctcatcttcccaccagctgctgatcaggtggcaactggaacagtcaccatcgtgtgcgtggctaacaagtacttcccggacgtgaccgtgacctgggaagtcgacggaaccactcagaccactggtatcgagaacagcaagacgccccagaactccgccgattgtacttataacctgtcctccacactgaccctcacctcgacccagtacaattcccacaaggagtacacttgcaaagtcacccagggaaccacttcagtggtgcagagcttcaaccggggggattgctga

SEQ ID NO: 24 - DNA, 1374 bp, synthetic construct
  source 1..1374: mol_type = other DNA
atggagactgggctgcgctggcttctcctggtcgctgtgctcaaaggtgtccagtgtcagtcggtggaggagtccaggggaggtctcttcaagccaacggagcccctgacactcacctgcacagcctctggattcaccatcagtagctaccacatgggctgggtccgccagactccagggaagcagctggagtggatcgggtggattggtagtagtggtgccacatactacgcgagctgggcgacaagccggtccaccatcaccagaaacaccaacgacaacacggtgactctgaaaatgaccagtctgacagccgcggacacggccacctatttctgtgcgagaagtggttggggtagttttgacatctggggcccaggcgccctggtcaccgtctcctcagggcaacctaaggctccatcagtcttcccactggccccctgctgcggggacacacccagctccacggtcaccctgggttgtcttgtgaagggatacctcccggaacccgtgaccgtgacctggaactccggcaccctgaccaatggagtgcggaccttcccgagcgtcaggcagtcctccgggttgtacagcttgtctagcgtggtgtccgtgacgtcgtcaagccagcctgtgacttgcaatgtggcccatccggccaccaacaccaaggtcgacaagaccgtggcgccttccacctgttccaagcccacttgcccgccgcctgagctcctgggaggaccgtccgtgttcatcttccctccaaaacccaaggataccctgatgattagccgcactcccgaagtcacttgcgtggtcgtggacgtgtcgcaggacgatcctgaggtgcagttcacttggtacatcaacaacgaacaagtccggacagctagaccaccgctgcgcgagcagcagttcaactcaactatccgggtggtgtccaccctgccgatcgcgcatcaggattggctgcgggggaaggagttcaagtgcaaagtccacaacaaggccctgcccgcccccatcgaaaagaccatctccaaggctcggggccagcctctggagcccaaagtgtacaccatgggcccgcctcgcgaggagctctcctcacgctcggtgtcgctgacttgcatgattaacggcttctacccttccgacatctccgtggaatgggagaagaacggaaaagccgaagataactacaagaccacgcccgccgtgctggactccgacggaagctatttcctgtactccaagctctccgtccccacttcggaatggcagaggggggacgtgttcacttgctccgtgatgcacgaggcactccacaaccactacacccaaaagagcatttcgcggtcacctggcaagtaa

SEQ ID NO: 25 - DNA, 1374 bp, synthetic construct
  source 1..1374: mol_type = other DNA
atggagactgggctgcgctggcttctcctggtcgctgtgctcaaaggtgtccagtgtcagtcggtgaaggagtccgagggaggtctcttcaagccaacggagcccctgacactcacctgcacagtctctggattctccctcagtagcgacaacatgggctgggtccgccagactccagggaagcagctggagtggatcgggtggattggtagtagtggtagcgcatactacgcgaggtgggcgaaaagccggtccaccatcaccagaaacaccaacgagaacacggtgactctgaaaatgaccagtctgacagccgcggacacggccacctatttctgtgcgagaagtggttggggtagttttgacatatggggcccaggcaccctggtcaccgtctcctcagggcaacctaaggctccatcagtcttcccactggccccctgctgcggggacacacccagctccacggtcaccctgggttgtcttgtgaagggatacctcccggaacccgtgaccgtgacctggaactccggcaccctgaccaatggagtgcggaccttcccgagcgtcaggcagtcctccgggttgtacagcttgtctagcgtggtgtccgtgacgtcgtcaagccagcctgtgacttgcaatgtggcccatccggccaccaacaccaaggtcgacaagaccgtggcgccttccacctgttccaagcccacttgcccgccgcctgagctcctgggaggaccgtccgtgttcatcttccctccaaaacccaaggataccctgatgattagccgcactcccgaagtcacttgcgtggtcgtggacgtgtcgcaggacgatcctgaggtgcagttcacttggtacatcaacaacgaacaagtccggacagctagaccaccgctgcgcgagcagcagttcaactcaactatccgggtggtgtccaccctgccgatcgcgcatcaggattggctgcgggggaaggagttcaagtgcaaagtccacaacaaggccctgcccgcccccatcgaaaagaccatctccaaggctcggggccagcctctggagcccaaagtgtacaccatgggcccgcctcgcgaggagctctcctcacgctcggtgtcgctgacttgcatgattaacggcttctacccttccgacatctccgtggaatgggagaagaacggaaaagccgaagataactacaagaccacgcccgccgtgctggactccgacggaagctatttcctgtactccaagctctccgtccccacttcggaatggcagaggggggacgtgttcacttgctccgtgatgcacgaggcactccacaaccactacacccaaaagagcatttcgcggtcacctggcaagtaa

SEQ ID NO: 26 - DNA, 711 bp, synthetic construct
  source 1..711: mol_type = other DNA
atggacacgagggcccccactcagctgctggggctcctgctgctctggctcccaggtgccacatttgcgcaagtgctgacccagactccagcctccgtgtctgccgctgtgggaggcacagtcaccatcaactgccagtccagtcagagtgtttataataacgaccgcttagcctggtttcagcagaaaccagggcagcctcccaagctcctgatctatctggcatccactctggcatctggggtcccatcgcggttcaaaggcagtggatctgggacacagttcactctcacaatcggcgaagtacagtgtgacgatgctgccacttactactgtcaaagctactataatggttatatttttggtttcggcggagggaccgaggtggtggtcaaaggtgatccagttgcacctactgtcctcatcttcccaccagctgctgatcaggtggcaactggaacagtcaccatcgtgtgcgtggctaacaagtacttcccggacgtgaccgtgacctgggaagtcgacggaaccactcagaccactggtatcgagaacagcaagacgccccagaactccgccgattgtacttataacctgtcctccacactgaccctcacctcgacccagtacaattcccacaaggagtacacttgcaaagtcacccagggaaccacttcagtggtgcagagcttcaaccggggggattgctga

SEQ ID NO: 27 - DNA, 711 bp, synthetic construct
  source 1..711: mol_type = other DNA
atggacacgagggcccccactcagctgctggggctcctgctgctctggctcccaggtgccacatttgcgcaagtgctgacccagactccatcccccgtgtctgcagctgtgggaagcacagtcaccatcagttgccagtccagtcagagtgtttatagtaacaaccgcttagcctggtttcaacagaaaccagggcagcctcccaagctcctgatctatctggcatccactctggcatctggggtcccatcgcggttcaaaggcagtggatctgggacacagttcactctcacaatcagcgaagtacagtgtgacgatgctgccacttactactgtcaaggctattatagtggttatatttttggtttcggcggagggaccgaggtggtagtcaaaggtgatccagttgcacctactgtcctcatcttcccaccagctgctgatcaggtggcaactggaacagtcaccatcgtgtgcgtggctaacaagtacttcccggacgtgaccgtgacctgggaagtcgacggaaccactcagaccactggtatcgagaacagcaagacgccccagaactccgccgattgtacttataacctgtcctccacactgaccctcacctcgacccagtacaattcccacaaggagtacacttgcaaagtcacccagggaaccacttcagtggtgcagagcttcaaccggggggattgctga

SEQ ID NO: 28 - protein, 16 aa, Phyllostomus discolor
SWKPGSRLQDVRSGPG

SEQ ID NO: 29 - protein, 16 aa, Phyllostomus hastatus
SWKPGTRLQDAPSDPG

SEQ ID NO: 30 - protein, 16 aa, Felis catus
SWKPRSQLQDAPSGPG

SEQ ID NO: 31 - protein, 16 aa, Equus caballus
SWKPCSQLQDAPSGPG

SEQ ID NO: 32 - protein, 16 aa, Panthera leo
SWKPRSQLQDTPSGPG

SEQ ID NO: 33 - protein, 16 aa, Nyctereutes procyonoides
SWKPRSWLQDAPSGPG

SEQ ID NO: 34 - protein, 16 aa, Lipotes vexillifer
SWKPRSHLQDAPSGPG

SEQ ID NO: 35 - protein, 16 aa, Pteronotus parnellii mesoamericanus
SWKPGSQLQDAPSGPG

SEQ ID NO: 36 - protein, 16 aa, Mus musculus
SWKPRSQLQDASSGPG

SEQ ID NO: 37 - protein, 16 aa, Mesocricetus auratus
SWKPHSHLQDTSSGPG

SEQ ID NO: 38 - protein, 16 aa, Microtus fortis
SWKPHPHLQDASSGPG

SEQ ID NO: 39 - protein, 16 aa, Cricetulus griseus
SWKSHSHLQDASSGPG

SEQ ID NO: 40 - protein, 16 aa, Mus pahari
SWKPRAQLQDASSGPG

SEQ ID NO: 41 - protein, 16 aa, Myodes glareolus
SWKPHSHLQDASSGPG

SEQ ID NO: 42 - protein, 16 aa, Onychomys torridus
SWKPHSQLQDASSGPG

SEQ ID NO: 43 - protein, 16 aa, Arvicanthis niloticus
SWKPRFQLQDASSGPG

SEQ ID NO: 44 - protein, 15 aa, Myotis myotis
SWKPRSQLQDAPSGP

SEQ ID NO: 45 - protein, 15 aa, Castor canadensis
SWKPRSQLQDVPSGP

SEQ ID NO: 46 - protein, 15 aa, Hyaena hyaena
SWKPHSQLQDVPSGP

SEQ ID NO: 47 - protein, 16 aa, Galemys pyrenaicus
SWKPRSQLQDAPTGPG

SEQ ID NO: 48 - protein, 15 aa, Neophocaena asiaeorientalis asiaeorientalis
WKPRSHLQDAPLGPG

SEQ ID NO: 49 - protein, 16 aa, Sousa chinensis
SWKPRSHLQDAPLGPG

SEQ ID NO: 50 - protein, 16 aa, Galemys pyrenaicus
SWKPRSQLQDAPTGPG

SEQ ID NO: 51 - protein, 16 aa, Bos taurus
SWKPHSHLQDAPVAPG

SEQ ID NO: 52 - protein, 16 aa, Ursus maritimus
SWKPHSQLQDAPSGAG

SEQ ID NO: 53 - protein, 16 aa, Ovis ammon polii x Ovis aries
SWKPHSQLQDAPVAPG

SEQ ID NO: 54 - protein, 16 aa, Peromyscus leucopus
SWKPHSQLQDASSEPG

SEQ ID NO: 55 - protein, 15 aa, Marmota monax
SWKPRSQLQDAPLGP

SEQ ID NO: 56 - protein, 14 aa, Grammomys surdaster
SWKPRSQLQDASSG

SEQ ID NO: 57 - protein, 15 aa, Ictidomys tridecemlineatus
SWKPRSQLQDEPLGP

SEQ ID NO: 58 - protein, 16 aa, Miniopterus natalensis
SWKPRSQLQDVPSAPG

SEQ ID NO: 59 - protein, 16 aa, Nannospalax galili
SWMPHSQLQDAPSGAG

SEQ ID NO: 60 - protein, 15 aa, Rattus norvegicus
SWKPRSQLQDASSGP

SEQ ID NO: 61 - protein, 15 aa, Ochotona princeps
SWRPHSQLQDAPSGP

SEQ ID NO: 62 - protein, 16 aa, Halichoerus grypus
SWRPRSQLQEAPSDPG

SEQ ID NO: 63 - protein, 16 aa, Odobenus rosmarus divergens
SWRPRSQMQEAPSGPG

SEQ ID NO: 64 - protein, 15 aa, Lontra canadensis
WKPGSRQQDAPSGPG

SEQ ID NO: 65 - protein, 15 aa, Lemur catta
SWKPRSQLPGAPSGP

SEQ ID NO: 66 - protein, 14 aa, Manis javanica
SWKPRSQLQEAPAG

SEQ ID NO: 67 - protein, 13 aa, Diceros bicornis minor
SWKPRSQVQDAPS

SEQ ID NO: 68 - protein, 29 aa, Canis lupus familiaris
QGPWMEEEEAAYGWMDFGRRSAEEGDQRP

SEQ ID NO: 69 - protein, 29 aa, Marmota marmota marmota
QEPWMEEEEAAYGWMDFGRRSAEEGDQRP

SEQ ID NO: 70 - protein, 29 aa, Sciurus carolinensis
QGPWMEEEEAAYGWMDFGRRSAEEADQRP

SEQ ID NO: 71 - protein, 29 aa, Nyctereutes procyonoides
QGPWMEEEEAAYGWMDFGRRSAEEEDQRP

SEQ ID NO: 72 - protein, 29 aa, Sciurus carolinensis
QGPWMEEEEAAYGWMDFGRRSAEEADQSP

SEQ ID NO: 73 - protein, 29 aa, Ictidomys tridecemlineatus
QGPWMEEEEAAYGWMDFGRRSAEEGDQHP

SEQ ID NO: 74 - protein, 29 aa, Urocitellus parryii
QGPWMEEEEAAYGWMDFGRRSAEEGDQXP

SEQ ID NO: 75 - protein, 29 aa, Sus scrofa
QGPWMEEEEEAYGWMDFGRRSAEEGDQRP

SEQ ID NO: 76 - protein, 29 aa, Halichoerus grypus
QGPWVEEEEAAYGWMDFGRRSAEEGDQRP

SEQ ID NO: 77 - protein, 28 aa, Tupaia chinensis
QGPWLEEEEAYGWMDFGRRSAEEGDQRP

SEQ ID NO: 78 - protein, 29 aa, Propithecus coquereli
QGPWLEEEEEAYGWMDFGRRSAEEGDQRP

SEQ ID NO: 79 - protein, 29 aa, Manis pentadactyla
QGPWLEEEEEAYGWMDFGRRSAEEEDQRP

SEQ ID NO: 80 - protein, 29 aa, Macaca nemestrina
QGPWMEEEEAAYGWMDFGRRSAEDENQQP

SEQ ID NO: 81 - protein, 26 aa, Mesocricetus auratus
PWMEEEEEAYGWMDFGRRSAEEGDQR

SEQ ID NO: 82 - protein, 28 aa, Castor canadensis
QGPWMEEEEEAYGWMDFGRRSAEEGDQR

SEQ ID NO: 83 - protein, 29 aa, Lemur catta
QGPWMEEEEEAYGWMDFGRRSAEEGDQHP

SEQ ID NO: 84 - protein, 28 aa, Echinops telfairi
QGPWMEEEEAYGWMDFGRRSAEEGDQQP

SEQ ID NO: 85 - protein, 29 aa, Otolemur garnettii
QGPWMEEEEEAYGWMDFGRRSAEEGNEHP

SEQ ID NO: 86 - protein, 29 aa, Orycteropus afer afer
QGPWMEEEEEAYGWMDFGRRSAEEMDERP

SEQ ID NO: 87 - protein, 28 aa, Bubalus bubalis
GPWVEEEEAAYGWMDFGRRSAEEGDQHP

SEQ ID NO: 88 - protein, 29 aa, Pteronotus parnellii mesoamericanus
QGPWLEEEEAAYGWMDFGRRSAEEGDQHP

SEQ ID NO: 89 - protein, 29 aa, Ursus maritimus
QGPWLEEEEAAYGWMDFGRRSAEEGDRRP

SEQ ID NO: 90 - protein, 29 aa, Moschus berezovskii
QGPWVEEEEAAYGWMDFGRRSAEEGDQHP

SEQ ID NO: 91 - protein, 29 aa, Ailuropoda melanoleuca
QGPWVEEEEAAYGWMDFGRRSAEEGDRHP

SEQ ID NO: 92 - protein, 29 aa, Gulo gulo
QGPWVEEEEAAYGWMDFGRRSAEEEDRRP

SEQ ID NO: 93 - protein, 29 aa, Leopardus geoffroyi
QGPWLEEEEAAYGWMDFGRRSAEDGDQHP

SEQ ID NO: 94 - protein, 29 aa, Dasypus novemcinctus
QGPWLEEEEAAYGWMDFGRRSAQDGDERP

SEQ ID NO: 95 - protein, 29 aa, Miniopterus natalensis
QGPWLEEEEDAYGWMDFGRRSAEEGDQHP

SEQ ID NO: 96 - protein, 29 aa, Molossus molossus
QGPWLEEEEEAYGWMDFGRRSAEEGDQHP

SEQ ID NO: 97 - protein, 29 aa, Myotis myotis
QGPWLEEEEEAYGWMDFGRRSAEEGDQQP

SEQ ID NO: 98 - protein, 29 aa, Dipodomys spectabilis
QGPWMQEEEEAYGWMDFGRRSAEEGDLRP

SEQ ID NO: 99 - protein, 29 aa, Eschrichtius robustus
QGPWVEEEEEAYGWMDFGRRSAEEGDLRP

SEQ ID NO: 100 - protein, 12 aa, synthetic construct
XSRLQDXPSGPG

SEQ ID NO: 101 - protein, 17 aa, synthetic construct
XWMEXEAAXAEEGDQRP

SEQ ID NO: 102 - protein, 76 aa, synthetic construct
SWKPRSRLQDAPSGPGANRGLEPHGLDQLGPASHHRRQLGLQGPPQLVADLSKKQGPWMEEEEAAYGWMDFGRRSA

SEQ ID NO: 103 - protein, 84 aa, synthetic construct
  MOD_RES 1: note = SUMO
HSWKPRSRLQDAPSGPGANRGLEPHGLDQLGPASHHRRQLGLQGPPQLVADLSKKQGPWMEEEEAAYGWMDFGRRSAEEGDQRP